European Patent Application EP 4 458 840 A1, published November 6, 2024. Title: Peptide having activities of skin condition improvement and uses thereof. Applicant: CAREGEN CO., LTD. The sequence listing filed with the application follows.

SEQUENCE LISTING (13 sequences)

SEQ ID NO: 1 - protein, 15 aa, Artificial Sequence
  Peptide 1
IHGTYKELLDTVTAP

SEQ ID NO: 2 - DNA, 20 bp, Artificial Sequence
  Col1a1_F
caccctcaagagcctgagtc

SEQ ID NO: 3 - DNA, 20 bp, Artificial Sequence
  Col1a1_R
agacggctgagtagggaaca

SEQ ID NO: 4 - DNA, 20 bp, Artificial Sequence
  Fibronectin_F
ccaggaaccgagtacaccat

SEQ ID NO: 5 - DNA, 20 bp, Artificial Sequence
  Fibronectin_R
atacccaggttgggtgatga

SEQ ID NO: 6 - DNA, 20 bp, Artificial Sequence
  Elastin_F
gcaagacctggctttggact

SEQ ID NO: 7 - DNA, 21 bp, Artificial Sequence
  Elastin_R
gggagtttctggttagggctg

SEQ ID NO: 8 - DNA, 20 bp, Artificial Sequence
  GAPDH_F
ggagccaaaagggtcatcat

SEQ ID NO: 9 - DNA, 20 bp, Artificial Sequence
  GAPDH_R
gtgatggcatggactgtggt

SEQ ID NO: 10 - DNA, 20 bp, Artificial Sequence
  SIRT1_F
tcagtggctggaacagtgag

SEQ ID NO: 11 - DNA, 20 bp, Artificial Sequence
  SIRT1_R
tctggcatgtcccactatca

SEQ ID NO: 12 - DNA, 20 bp, Artificial Sequence
  AQP3_F
ccttcttgggtgctggaata

SEQ ID NO: 13 - DNA, 20 bp, Artificial Sequence
  AQP3_R
acacgataagggaggctgtg